European Patent Application EP 4 748 391 A1, published May 27, 2026. Title: IMMUNOGENIC COMPLEX. Applicant: MINERVAX APS. The sequence listing filed with the application follows.

SEQUENCE LISTING (22 sequences)

SEQ ID NO: 1 - DNA, 537 bp, synthetic construct
  source 1..537: mol_type = other DNA
gggcccctgggatccgctgaagtaatttcaggaagtgctgttacgttaaacacaaatatgactaaaaatgttcagaatggtagagcatatatagatttatatgatgtgaaaaatgggaaaatagatccattacaattaattacgttaaattcacctgatttaaaagctcagtatgtcattaggcaaggcggcaattatttcacacaaccttctgaattgactactgttggtgcagctagtattaattatacagtattgaagacagatggaagtcctcatacgaagcctgatggacaagtggatattataaacgtttcattgactatttacaattcttcagctttgagagataaaatagatgaagttaaaaagaaagcggaagaccctaaatgggacgagggaagtcgcgataaagttttgataagtttagatgatatcaaaacagatattgataataatcctaagacgcaatcagacattgccaataaaataactgaagttactaatttagaaaaaatactagtacctcgaatccca

SEQ ID NO: 2 - protein, 179 aa, synthetic construct
GPLGSAEVISGSAVTLNTNMTKNVQNGRAYIDLYDVKNGKIDPLQLITLNSPDLKAQYVIRQGGNYFTQPSELTTVGAASINYTVLKTDGSPHTKPDGQVDIINVSLTIYNSSALRDKIDEVKKKAEDPKWDEGSRDKVLISLDDIKTDIDNNPKTQSDIANKITEVTNLEKILVPRIP

SEQ ID NO: 3 - DNA, 525 bp, synthetic construct
  source 1..525: mol_type = other DNA
gggcccctgggatcctctacaattccagggagtgcagcgaccttaaatacaagcatcactaaaaatatacaaaacggaaatgcttacatagatttatatgatgtaaaattaggtaaaatagatccattacaattaattgttttagaacaaggttttacagcaaagtatgtttttagacaaggtactaaatactatggggatgtttctcagttgcagagtacaggaagggctagtcttacctataatatatttggtgaagatggactaccacatgtaaagactgatggacaaattgatatagttagtgttgctttaactatttatgattcaacaaccttgagggataagattgaagaagttagaacgaatgcaaacgatcctaagtggacggaagaaagtcgtactgaggttttaacaggattagatacaattaagacagatattgataataatcctaagacgcaaacagatattgatagtaaaattgttgaggttaatgaattagagaaattgttagtattgtca

SEQ ID NO: 4 - protein, 175 aa, synthetic construct
GPLGSSTIPGSAATLNTSITKNIQNGNAYIDLYDVKLGKIDPLQLIVLEQGFTAKYVFRQGTKYYGDVSQLQSTGRASLTYNIFGEDGLPHVKTDGQIDIVSVALTIYDSTTLRDKIEEVRTNANDPKWTEESRTEVLTGLDTIKTDIDNNPKTQTDIDSKIVEVNELEKLLVLS

SEQ ID NO: 5 - DNA, 1053 bp, synthetic construct
  source 1..1053: mol_type = other DNA
gggcccctgggatccgctgaagtaatttcaggaagtgctgttacgttaaacacaaatatgactaaaaatgttcagaatggtagagcatatatagatttatatgatgtgaaaaatgggaaaatagatccattacaattaattacgttaaattcacctgatttaaaagctcagtatgtcattaggcaaggcggcaattatttcacacaaccttctgaattgactactgttggtgcagctagtattaattatacagtattgaagacagatggaagtcctcatacgaagcctgatggacaagtggatattataaacgtttcattgactatttacaattcttcagctttgagagataaaatagatgaagttaaaaagaaagcggaagaccctaaatgggacgagggaagtcgcgataaagttttgataagtttagatgatatcaaaacagatattgataataatcctaagacgcaatcagacattgccaataaaataactgaagttactaatttagaaaaaatactagtacctcgaatcccagaattctctacaattccagggagtgcagcgaccttaaatacaagcatcactaaaaatatacaaaacggaaatgcttacatagatttatatgatgtaaaattaggtaaaatagatccattacaattaattgttttagaacaaggttttacagcaaagtatgtttttagacaaggtactaaatactatggggatgtttctcagttgcagagtacaggaagggctagtcttacctataatatatttggtgaagatggactaccacatgtaaagactgatggacaaattgatatagttagtgttgctttaactatttatgattcaacaaccttgagggataagattgaagaagttagaacgaatgcaaacgatcctaagtggacggaagaaagtcgtactgaggttttaacaggattagatacaattaagacagatattgataataatcctaagacgcaaacagatattgatagtaaaattgttgaggttaatgaattagagaaattgttagtattgtca

SEQ ID NO: 6 - protein, 378 aa, synthetic construct
GPLGSASVLIGISFLGGFTQGQFNISTDTVFAAEVISGSAVTLNTNMTKNVQNGRAYIDLYDVKNGKIDPLQLITLNSPDLKAQYVIRQGGNYFTQPSELTTVGAASINYTVLKTDGSPHTKPDGQVDIINVSLTIYNSSALRDKIDEVKKKAEDPKWDEGSRDKVLISLDDIKTDIDNNPKTQSDIANKITEVTNLEKILVPRIPEFSTIPGSAATLNTSITKNIQNGNAYIDLYDVKLGKIDPLQLIVLEQGFTAKYVFRQGTKYYGDVSQLQSTGRASLTYNIFGEDGLPHVKTDGQIDIVSVALTIYDSTTLRDKIEEVRTNANDPKWTEESRTEVLTGLDTIKTDIDNNPKTQTDIDSKIVEVNELEKLLVLS

SEQ ID NO: 7 - DNA, 525 bp, synthetic construct
  source 1..525: mol_type = other DNA
atggccgaagttattagcggtagcgcagcaaccctgaatagcgcactggttaaaaatgttagcggtggcaaagcctatatcgacatctatgatgtgaaaaacggcaaaattgatccgctgaatctgattgttctgcctccgagcaattatagcgccaactattatatcaaacagggtggtcgcattttcaccaatgttaatcagctgcagacaccgggtacagcaaccattacctataacattctggatgaaaatggcaacccgtataccaaaagtgatggccagattgatattgttagcctggttaccaccgtttatgataccaccgaactgcgcaataacatcaacaaagttattgagaatgccaacgacccgaaatggtcagatgatagccgtaaagatgttctgagcaaaatcgaggtgatcaaaaacgatattgataacaacccgaaaacccagagcgatatcgacaacaaaattgtggaagtgaacgagctggaaaaactgctggttctgccgtaataa

SEQ ID NO: 8 - protein, 173 aa, synthetic construct
MAEVISGSAATLNSALVKNVSGGKAYIDIYDVKNGKIDPLNLIVLTPSNYSANYYIKQGGRIFTSVNQLQTPGTATITYNILDENGNPYTKSDGQIDIVSLVTTVYDTTELRNNINKVIENANDPKWSDDSRKDVLSKIEVIKNDIDNNPKTQSDIDNKIVEVNELEKLLVLP

SEQ ID NO: 9 - DNA, 528 bp, synthetic construct
  source 1..528: mol_type = other DNA
atggcaagcaccattccgggtagcgcagcaaccctgaataccagcattaccaaaaacattcagaatggcaacgcctatatcgatctgtatgatgtgaaaaacggtctgattgatccgcagaatctgattgttctgaatccgagcagctatagcgccaactattatatcaaacagggtgccaaatattacagcaacccgagcgaaattaccaccaccggtagcgcaaccattacctttaacattctggatgaaaccggcaacccgcataaaaaagcagatggtcagattgatattgtgagcgttaacctgaccatttatgatagcaccgcactgcgtaatcgtattgatgaagttattaacaatgccaacgacccgaaatggtctgatggtagccgtgatgaagtgctgaccggtctggaaaaaatcaaaaaagatatcgataacaacccgaaaacccagatcgacattgacaacaaaattaacgaagtgaacgaaatcgaaaaactgctggttgttagcctgtaataa

SEQ ID NO: 10 - protein, 173 aa, synthetic construct
ASTIPGSAATLNTSITKNIQNGNAYIDLYDVKNGLIDPQNLIVLNPSSYSANYYIKQGAKYYSNPSEITTTGSATITFNILDETGNPHKKADGQIDIVSVNLTIYDSTALRNRIDEVINNANDPKWSDGSRDEVLTGLEKIKKDIDNNPKTQIDIDNKINEVNEIEKLLVVSL

SEQ ID NO: 11 - DNA, 1047 bp, synthetic construct
  source 1..1047: mol_type = other DNA
atggccgaagttattagcggtagcgcagcaaccctgaatagcgcactggttaaaaatgttagcggtggcaaagcctatatcgacatctatgatgtgaaaaacggcaaaattgatccgctgaatctgattgttctgcctccgagcaattatagcgccaactattatatcaaacagggtggtcgcattttcaccaatgttaatcagctgcagacaccgggtacagcaaccattacctataacattctggatgaaaatggcaacccgtataccaaaagtgatggccagattgatattgttagcctggttaccaccgtttatgataccaccgaactgcgcaataacatcaacaaagttattgagaatgccaacgacccgaaatggtcagatgatagccgtaaagatgttctgagcaaaatcgaggtgatcaaaaacgatattgataacaacccgaaaacccagagcgatatcgacaacaaaattgtggaagtgaacgagctggaaaaactgctggttctgccggaatttagcaccattccgggttcagcagccacactgaataccagcattaccaaaaacattcagaatggcaacgcctacattgatctgtacgatgtaaaaaatggtctgatcgatccgcagaacctgatcgtgctgaatccgagcagctattcagccaattattatattaaacaaggcgcaaaatactatagcaacccgagcgaaattaccaccaccggtagcgccaccattacgtttaatatcctggacgaaaccggtaacccgcataaaaaagcagatggtcaaattgatatcgtgagcgttaacctgacgatttatgatagcacagccctgcgtaatcgtattgatgaagtgattaataacgcgaatgatcctaaatggtccgatggtagtcgtgatgaagtactgaccggtctggaaaaaatcaaaaaagacatcgacaataatccgaaaacgcagattgacattgacaataaaatcaacgaggtgaacgagatcgagaaactgctggtagttagcctgtaataa

SEQ ID NO: 12 - protein, 347 aa, synthetic construct
MAEVISGSAATLNSALVKNVSGGKAYIDIYDVKNGKIDPLNLIVLTPSNYSANYYIKQGGRIFTSVNQLQTPGTATITYNILDENGNPYTKSDGQIDIVSLVTTVYDTTELRNNINKVIENANDPKWSDDSRKDVLSKIEVIKNDIDNNPKTQSDIDNKIVEVNELEKLLVLPEFSTIPGSAATLNTSITKNIQNGNAYIDLYDVKNGLIDPQNLIVLNPSSYSANYYIKQGAKYYSNPSEITTTGSATITFNILDETGNPHKKADGQIDIVSVNLTIYDSTALRNRIDEVINNANDPKWSDGSRDEVLTGLEKIKKDIDNNPKTQIDIDNKINEVNEIEKLLVVSL

SEQ ID NO: 13 - DNA, 310 bp, synthetic construct
  source 1..310: mol_type = other DNA
gtagttgaaggaagtgctgcaacattaaatactgccatgactaaaaacatgcagaatgggaatgcatatattgatatttatgatgttaaattaggaaaaattgatccattacaactgattaaattggaaccgggatacactgctatttattacattacacaaggttcaaaagtttatgcaaatgtttcggagctacaaacaccaggagcagcgaaagttaattatcgtattcaaacctctgatggaagcgatcatataaaatctgatggtcaattagacagcgttaatatttcattaacagtttatgatt

SEQ ID NO: 14 - protein, 103 aa, synthetic construct
VVEGSAATLNTAMTKNMQNGNAYIDIYDVKLGKIDPLQLIKLEPGYTAIYYITQGSKVYANVSELQTPGAAKVNYRIQTSDGSDHIKSDGQLDSVNISLTVYD

SEQ ID NO: 15 - DNA, 525 bp, synthetic construct
  source 1..525: mol_type = other DNA
atggctgaagtaatttcaggaagtgctgttacgttaaacacaaatatgactaaaaatgttcagaatggtagagcatatatagatttatatgatgtgaaaaatgggaaaatagatccattacaattaattacgttaaattcacctgatttaaaagctcagtatgtcattaggcaaggcggcaattatttcacacaaccttctgaattgactactgttggtgcagctagtattaattatacagtattgaagacagatggaagtcctcatacgaagcctgatggacaagtggatattataaacgtttcattgactatttacaattcttcagctttgagagataaaatagatgaagttaaaaagaaagcggaagaccctaaatgggacgagggaagtcgcgataaagttttgataagtttagatgatatcaaaacagatattgataataatcctaagacgcaatcagacattgccaataaaataactgaagttactaatttagaaaaaatactagtacctcgaatccca

SEQ ID NO: 16 - protein, 175 aa, synthetic construct
MAEVISGSAVTLNTNMTKNVQNGRAYIDLYDVKNGKIDPLQLITLNSPDLKAQYVIRQGGNYFTQPSELTTVGAASINYTVLKTDGSPHTKPDGQVDIINVSLTIYNSSALRDKIDEVKKKAEDPKWDEGSRDKVLISLDDIKTDIDNNPKTQSDIANKITEVTNLEKILVPRIP

SEQ ID NO: 17 - DNA, 516 bp, synthetic construct
  source 1..516: mol_type = other DNA
tctacaattccagggagtgcagcgaccttaaatacaagcatcactaaaaatatacaaaacggaaatgcttacatagatttatatgatgtaaaattaggtaaaatagatccattacaattaattgttttagaacaaggttttacagcaaagtatgtttttagacaaggtactaaatactatggggatgtttctcagttgcagagtacaggaagggctagtcttacctataatatatttggtgaagatggactaccacatgtaaagactgatggacaaattgatatagttagtgttgctttaactatttatgattcaacaaccttgagggataagattgaagaagttagaacgaatgcaaacgatcctaagtggacggaagaaagtcgtactgaggttttaacaggattagatacaattaagacagatattgataataatcctaagacgcaaacagatattgatagtaaaattgttgaggttaatgaattagagaaattgttagtattgtcataataa

SEQ ID NO: 18 - protein, 170 aa, synthetic construct
STIPGSAATLNTSITKNIQNGNAYIDLYDVKLGKIDPLQLIVLEQGFTAKYVFRQGTKYYGDVSQLQSTGRASLTYNIFGEDGLPHVKTDGQIDIVSVALTIYDSTTLRDKIEEVRTNANDPKWTEESRTEVLTGLDTIKTDIDNNPKTQTDIDSKIVEVNELEKLLVLS

SEQ ID NO: 19 - DNA, 522 bp, synthetic construct
  source 1..522: mol_type = other DNA
agcaccattccgggttcagcagccacactgaataccagcattaccaaaaacattcagaatggcaacgcctacattgatctgtacgatgtaaaaaatggtctgatcgatccgcagaacctgatcgtgctgaatccgagcagctattcagccaattattatattaaacaaggcgcaaaatactatagcaacccgagcgaaattaccaccaccggtagcgccaccattacgtttaatatcctggacgaaaccggtaacccgcataaaaaagcagatggtcaaattgatatcgtgagcgttaacctgacgatttatgatagcacagccctgcgtaatcgtattgatgaagtgattaataacgcgaatgatcctaaatggtccgatggtagtcgtgatgaagtactgaccggtctggaaaaaatcaaaaaagacatcgacaataatccgaaaacgcagattgacattgacaataaaatcaacgaggtgaacgagatcgagaaactgctggtagttagcctgtaataa

SEQ ID NO: 20 - protein, 172 aa, synthetic construct
STIPGSAATLNTSITKNIQNGNAYIDLYDVKNGLIDPQNLIVLNPSSYSANYYIKQGAKYYSNPSEITTTGSATITFNILDETGNPHKKADGQIDIVSVNLTIYDSTALRNRIDEVINNANDPKWSDGSRDEVLTGLEKIKKDIDNNPKTQIDIDNKINEVNEIEKLLVVSL

SEQ ID NO: 21 - DNA, 1047 bp, synthetic construct
  source 1..1047: mol_type = other DNA
atggctgaagtaatttcaggaagtgctgttacgttaaacacaaatatgactaaaaatgttcagaatggtagagcatatatagatttatatgatgtgaaaaatgggaaaatagatccattacaattaattacgttaaattcacctgatttaaaagctcagtatgtcattaggcaaggcggcaattatttcacacaaccttctgaattgactactgttggtgcagctagtattaattatacagtattgaagacagatggaagtcctcatacgaagcctgatggacaagtggatattataaacgtttcattgactatttacaattcttcagctttgagagataaaatagatgaagttaaaaagaaagcggaagaccctaaatgggacgagggaagtcgcgataaagttttgataagtttagatgatatcaaaacagatattgataataatcctaagacgcaatcagacattgccaataaaataactgaagttactaatttagaaaaaatactagtacctcgaatcccagaattctctacaattccagggagtgcagcgaccttaaatacaagcatcactaaaaatatacaaaacggaaatgcttacatagatttatatgatgtaaaattaggtaaaatagatccattacaattaattgttttagaacaaggttttacagcaaagtatgtttttagacaaggtactaaatactatggggatgtttctcagttgcagagtacaggaagggctagtcttacctataatatatttggtgaagatggactaccacatgtaaagactgatggacaaattgatatagttagtgttgctttaactatttatgattcaacaaccttgagggataagattgaagaagttagaacgaatgcaaacgatcctaagtggacggaagaaagtcgtactgaggttttaacaggattagatacaattaagacagatattgataataatcctaagacgcaaacagatattgatagtaaaattgttgaggttaatgaattagagaaattgttagtattgtcataataa

SEQ ID NO: 22 - protein, 347 aa, synthetic construct
MAEVISGSAVTLNTNMTKNVQNGRAYIDLYDVKNGKIDPLQLITLNSPDLKAQYVIRQGGNYFTQPSELTTVGAASINYTVLKTDGSPHTKPDGQVDIINVSLTIYNSSALRDKIDEVKKKAEDPKWDEGSRDKVLISLDDIKTDIDNNPKTQSDIANKITEVTNLEKILVPRIPEFSTIPGSAATLNTSITKNIQNGNAYIDLYDVKLGKIDPLQLIVLEQGFTAKYVFRQGTKYYGDVSQLQSTGRASLTYNIFGEDGLPHVKTDGQIDIVSVALTIYDSTTLRDKIEEVRTNANDPKWTEESRTEVLTGLDTIKTDIDNNPKTQTDIDSKIVEVNELEKLLVLS